European Patent Application EP 4 692 108 A1, published February 11, 2026. Title: Peptide promoting hair growth or inhibiting hair loss and uses thereof. Applicant: CAREGEN CO., LTD. Application KR. The sequence listing filed with the application follows.

SEQUENCE LISTING (26 sequences)

SEQ ID NO: 1 - protein, 10 aa, synthetic construct
RQTRVERSHS

SEQ ID NO: 2 - DNA, 20 bp, synthetic construct
  source 1..20: mol_type = other DNA
ccagctattgtaacacctca

SEQ ID NO: 3 - DNA, 20 bp, synthetic construct
  source 1..20: mol_type = other DNA
ttcagatgtaggcagctgtc

SEQ ID NO: 4 - DNA, 25 bp, synthetic construct
  source 1..25: mol_type = other DNA
accagcagcgactctgaggaggaac

SEQ ID NO: 5 - DNA, 26 bp, synthetic construct
  source 1..26: mol_type = other DNA
tgaccctcttggcagcaggatagtcc

SEQ ID NO: 6 - DNA, 28 bp, synthetic construct
  source 1..28: mol_type = other DNA
accttcgttgccctctgtgccacagatg

SEQ ID NO: 7 - DNA, 21 bp, synthetic construct
  source 1..21: mol_type = other DNA
aggcccggaggcagtccgggt

SEQ ID NO: 8 - DNA, 20 bp, synthetic construct
  source 1..20: mol_type = other DNA
ggagccaaaagggtcatcat

SEQ ID NO: 9 - DNA, 20 bp, synthetic construct
  source 1..20: mol_type = other DNA
gtgatggcatggactgtggt

SEQ ID NO: 10 - DNA, 20 bp, synthetic construct
  source 1..20: mol_type = other DNA
ctgcatgcaagagtgacacc

SEQ ID NO: 11 - DNA, 20 bp, synthetic construct
  source 1..20: mol_type = other DNA
gacattgccccttccctttg

SEQ ID NO: 12 - DNA, 20 bp, synthetic construct
  source 1..20: mol_type = other DNA
aagctgcaacgaaaacgacg

SEQ ID NO: 13 - DNA, 20 bp, synthetic construct
  source 1..20: mol_type = other DNA
ggtggggctagtcaagtctg

SEQ ID NO: 14 - DNA, 20 bp, synthetic construct
  source 1..20: mol_type = other DNA
ccagcaagacggagatcaca

SEQ ID NO: 15 - DNA, 20 bp, synthetic construct
  source 1..20: mol_type = other DNA
gaagaggcttccctgatggc

SEQ ID NO: 16 - DNA, 20 bp, synthetic construct
  source 1..20: mol_type = other DNA
cctatccccgggactaagac

SEQ ID NO: 17 - DNA, 20 bp, synthetic construct
  source 1..20: mol_type = other DNA
atgctcttcaggggcaacac

SEQ ID NO: 18 - DNA, 20 bp, synthetic construct
  source 1..20: mol_type = other DNA
cagtggaatctgcatccccg

SEQ ID NO: 19 - DNA, 19 bp, synthetic construct
  source 1..19: mol_type = other DNA
cagcgatgctctgttgtgg

SEQ ID NO: 20 - DNA, 20 bp, synthetic construct
  source 1..20: mol_type = other DNA
ccgttctccccaggaaactt

SEQ ID NO: 21 - DNA, 20 bp, synthetic construct
  source 1..20: mol_type = other DNA
tgcagcgatcaggtcgttta

SEQ ID NO: 22 - DNA, 20 bp, synthetic construct
  source 1..20: mol_type = other DNA
tggaccagctaaccaacgac

SEQ ID NO: 23 - DNA, 20 bp, synthetic construct
  source 1..20: mol_type = other DNA
gtcattgttccggttggcag

SEQ ID NO: 24 - DNA, 20 bp, synthetic construct
  source 1..20: mol_type = other DNA
cccagccaacctatgaggag

SEQ ID NO: 25 - DNA, 20 bp, synthetic construct
  source 1..20: mol_type = other DNA
cttgaggagaccagcaccac

SEQ ID NO: 26 - protein, 10 aa, synthetic construct
RQTRVQRSHS